European Patent Specification EP 3 589 739 B1, published July 15, 2026. Title: COMPOSITIONS USEFUL IN TREATMENT OF SPINAL MUSCULAR ATROPHY. Applicant: The Trustees of the University of Pennsylvania. The sequence listing filed with the application follows.

SEQUENCE LISTING (26 sequences)

SEQ ID NO: 1 - DNA, 882 bp, Artificial Sequence
  engineered sequence encoding human SMN variant D protein
  CDS (1)..(882)
atggccatgtcgagtgggggcagtggagggggagtgccagaacaggaagattccgtgctgttcaggcgaggaaccgggcagagtgacgacagtgacatttgggacgacacggccctgatcaaggcctatgacaaagccgtggcctccttcaagcacgcgctgaagaacggcgacatttgcgaaaccagcggcaagcctaagaccacccctaaacggaagcccgccaagaaaaataagtcccagaaaaagaacacagccgcaagtcttcagcaatggaaggtgggggataagtgctccgcgatatggagtgaagacgggtgcatctatcctgccaccatcgccagcatagacttcaagcgcgaaacctgcgtggtggtgtacactggatacgggaaccgggaggagcagaacctgagcgacctgttgagccctatttgtgaggtggccaacaacatcgagcagaatgcgcaagaaaatgaaaacgagagtcaggtgtccaccgatgagagtgaaaacagtaggagccccggcaacaaatccgacaatatcaagcccaaaagcgcaccctggaatagcttccttccacccccccccccaatgcccggacctcgactgggccccggaaagcctggcctgaagttcaacggcccccctcctcctcctccccctcctcccccccacctgctgagctgctggttgccccctttcccttcgggaccccctatcatacctccccccccccctatttgccctgactccctggacgacgcggacgcgctgggcagtatgctcatctcgtggtacatgtcaggataccacaccgggtactacatgggcttcagacaaaatcagaaggaaggacgatgtagtcactccctgaat

SEQ ID NO: 2 - protein, 294 aa, Artificial Sequence
  Synthetic Construct
MAMSSGGSGGGVPEQEDSVLFRRGTGQSDDSDIWDDTALIKAYDKAVASFKHALKNGDICETSGKPKTTPKRKPAKKNKSQKKNTAASLQQWKVGDKCSAIWSEDGCIYPATIASIDFKRETCVVVYTGYGNREEQNLSDLLSPICEVANNIEQNAQENENESQVSTDESENSRSPGNKSDNIKPKSAPWNSFLPPPPPMPGPRLGPGKPGLKFNGPPPPPPPPPPHLLSCWLPPFPSGPPIIPPPPPICPDSLDDADALGSMLISWYMSGYHTGYYMGFRQNQKEGRCSHSLN

SEQ ID NO: 3 - DNA, 874 bp, Homo sapiens
cagcggcggcagtggtggcggcgtcccggagcaggaggattccgtgctgttccggcgcggcacaggccagagcgatgattctgacatttgggatgatacagcactgataaaagcatatgataaagctgtggcttcatttaagcatgctctaaagaatggtgacatttgtgaaacttcgggtaaaccaaaaaccacacctaaaagaaaacctgctaagaagaataaaagccaaaagaagaatactgcagcttccttacaacagtggaaagttggggacaaatgttctgccatttggtcagaagacggttgcatttacccagctaccattgcttcaattgattttaagagagaaacctgtgttgtggtttacactggatatggaaatagagaggagcaaaatctgtccgatctactttccccaatctgtgaagtagctaataatatagaacagaatgctcaagagaatgaaaatgaaagccaagtttcaacagatgaaagtgagaactccaggtctcctggaaataaatcagataacatcaagcccaaatctgctccatggaactcttttctccctccaccaccccccatgccagggccaagactgggaccaggaaagccaggtctaaaattcaatggcccaccaccgccaccgccaccaccaccaccccacttactatcatgctggctgcctccatttccttctggaccaccaataattcccccaccacctcccatatgtccagattctcttgatgatgctgatgctttgggaagtatgttaatttcatggtacatgagtggctatcatactggctattatatgggtttcagacaaaatcaaaaagaaggaaggtgctcacattccttaaattaa

SEQ ID NO: 4 - DNA, 885 bp, Artificial Sequence
  Engineered hSMN transgene G2
atggcgatgagcagcggcggcagtggtggcggcgtcccggagcaggaggattccgtgctgttccggcgcggcacaggccagagcgatgattctgacatttgggatgatacagcactgataaaagcatatgataaagctgtggcttcatttaagcatgctctaaagaatggtgacatttgtgaaacttcgggtaaaccaaaaaccacacctaaaagaaaacctgctaagaagaataaaagccaaaagaagaatactgcagcttccttacaacagtggaaagttggggacaaatgttctgccatttggtcagaagacggttgcatttacccagctaccattgcttcaattgattttaagagagaaacctgtgttgtggtttacactggatatggaaatagagaggagcaaaatctgtccgatctactttccccaatctgtgaagtagctaataatatagaacagaatgctcaagagaatgaaaatgaaagccaagtttcaacagatgaaagtgagaactccaggtctcctggaaataaatcagataacatcaagcccaaatctgctccatggaactcttttctccctccaccaccccccatgccagggccaagactgggaccaggaaagccaggtctaaaattcaatggcccaccaccgccaccgccaccaccaccaccccacttactatcatgctggctgcctccatttccttctggaccaccaataattcccccaccacctcccatatgtccagattctcttgatgatgctgatgctttgggaagtatgttaatttcatggtacatgagtggctatcatactggctattatatgggtttcagacaaaatcaaaaagaaggaaggtgctcacattccttaaattaa

SEQ ID NO: 5 - DNA, 885 bp, Artificial Sequence
  Engineered SMN transgene G3
atggctatgagcagtggcggctctggcggcggagtgcctgagcaggaagatagcgtgctgttcagacggggcaccggccagagcgacgacagcgacatctgggatgacaccgccctgatcaaggcctacgacaaggccgtggccagcttcaagcacgccctgaagaacggcgatatctgcgagacaagcggcaagcccaagaccacccccaagagaaagcccgccaagaagaacaagagccagaagaagaataccgccgcctccctgcagcagtggaaagtgggcgataagtgcagcgccatttggagcgaggacggctgcatctaccccgccacaatcgccagcatcgacttcaagcgggaaacctgcgtggtggtgtacacaggctacggcaacagagaggaacagaacctgagcgacctgctgagccccatctgcgaggtggccaacaacatcgagcagaacgcccaggaaaacgagaacgagtcccaggtgtccaccgacgagagcgagaacagcagaagccccggcaacaagagcgacaacatcaagcctaagagcgccccctggaacagcttcctgcctccccctccaccaatgcctggccctagactgggacctggcaagcccggcctgaagttcaatggccctcctcccccacctccaccaccaccccctcatctgctgagctgttggctgcccccattccctagcggccctcccatcattcctccaccccccccaatctgccccgacagcctggatgatgctgatgccctgggctccatgctgatctcttggtacatgagcggctaccacaccggctactacatgggcttccggcagaaccagaaagagggccgctgtagccacagcctgaactga

SEQ ID NO: 6 - DNA, 885 bp, Artificial Sequence
  Engineered SMN transgene G4
atggcgatgagcagcggtggttccggaggaggggtgccggagcaggaggattccgtccttttcagacggggaaccggccagtcggacgactcggacatctgggatgacaccgcactgatcaaagcatacgataaagcagtggcatcgttcaagcacgcccttaagaatggagacatttgcgaaaccagcgggaagccaaaaactactccgaagcgcaagcccgccaagaagaataagtcacagaagaaaaacaccgccgcttcgctgcaacagtggaaagtgggcgacaagtgctccgcgatctggtcagaggatggctgcatctacccggccacgatcgcctccatcgacttcaagcgggaaacttgtgtggtcgtctacactggctacggaaaccgcgaggaacagaatctcagcgatctcctcagcccgatttgtgaggtggccaacaatatcgaacagaacgcgcaagaaaacgagaacgagtcccaagtgtcgactgacgaatcggaaaattcgcgctcaccaggaaacaagtcagataacatcaagcccaaaagcgcgccatggaacagctttttgccgccaccaccacctatgcctggaccgaggctgggaccgggaaagccgggactcaaattcaacggcccaccgcctccgccacctccgcctccaccccacttgctgtcctgctggctgccgccatttccgtcgggtccgcctatcatccctcctccaccgccgatttgccccgactcactcgacgatgctgacgccctggggtcaatgctgatctcctggtatatgtccggctaccataccggatactacatgggattccggcagaaccaaaaggaagggagatgctcccattcgctgaattga

SEQ ID NO: 7 - DNA, 2211 bp, Artificial Sequence
  AAVhu68 vp1 coding sequence
  CDS (1)..(2211): AAVhu68 vp1
atggctgccgatggttatcttccagattggctcgaggacaacctcagtgaaggcattcgcgagtggtgggctttgaaacctggagcccctcaacccaaggcaaatcaacaacatcaagacaacgctcggggtcttgtgcttccgggttacaaataccttggacccggcaacggactcgacaagggggagccggtcaacgaagcagacgcggcggccctcgagcacgacaaggcctacgaccagcagctcaaggccggagacaacccgtacctcaagtacaaccacgccgacgccgagttccaggagcggctcaaagaagatacgtcttttgggggcaacctcgggcgagcagtcttccaggccaaaaagaggcttcttgaacctcttggtctggttgaggaagcggctaagacggctcctggaaagaagaggcctgtagagcagtctcctcaggaaccggactcctccgtgggtattggcaaatcgggtgcacagcccgctaaaaagagactcaatttcggtcagactggcgacacagagtcagtccccgaccctcaaccaatcggagaacctcccgcagccccctcaggtgtgggatctcttacaatggcttcaggtggtggcgcaccagtggcagacaataacgaaggtgccgatggagtgggtagttcctcgggaaattggcattgcgattcccaatggctgggggacagagtcatcaccaccagcacccgaacctgggccctgcccacctacaacaatcacctctacaagcaaatctccaacagcacatctggaggatcttcaaatgacaacgcctacttcggctacagcaccccctgggggtattttgacttcaacagattccactgccacttctcaccacgtgactggcaaagactcatcaacaacaactggggattccggcctaagcgactcaacttcaagctcttcaacattcaggtcaaagaggttacggacaacaatggagtcaagaccatcgctaataaccttaccagcacggtccaggtcttcacggactcagactatcagctcccgtacgtgctcgggtcggctcacgagggctgcctcccgccgttcccagcggacgttttcatgattcctcagtacgggtatctaacgcttaatgatggaagccaagccgtgggtcgttcgtccttttactgcctggaatatttcccgtcgcaaatgctaagaacgggtaacaacttccagttcagctacgagtttgagaacgtacctttccatagcagctatgctcacagccaaagcctggaccgactcatgaatccactcatcgaccaatacttgtactatctctcaaagactattaacggttctggacagaatcaacaaacgctaaaattcagtgtggccggacccagcaacatggctgtccagggaagaaactacatacctggacccagctaccgacaacaacgtgtctcaaccactgtgactcaaaacaacaacagcgaatttgcttggcctggagcttcttcttgggctctcaatggacgtaatagcttgatgaatcctggacctgctatggccagccacaaagaaggagaggaccgtttctttcctttgtctggatctttaatttttggcaaacaaggaactggaagagacaacgtggatgcggacaaagtcatgataaccaacgaagaagaaattaaaactaccaacccagtagcaacggagtcctatggacaagtggccacaaaccaccagagtgcccaagcacaggcgcagaccggctgggttcaaaaccaaggaatacttccgggtatggtttggcaggacagagatgtgtacctgcaaggacccatttgggccaaaattcctcacacggacggcaactttcacccttctccgctgatgggagggtttggaatgaagcacccgcctcctcagatcctcatcaaaaacacacctgtacctgcggatcctccaacggctttcaacaaggacaagctgaactctttcatcacccagtattctactggccaagtcagcgtggagattgagtgggagctgcagaaggaaaacagcaagcgctggaacccggagatccagtacacttccaactattacaagtctaataatgttgaatttgctgttaatactgaaggtgtttattctgaaccccgccccattggcaccagatacctgactcgtaatctgtaa

SEQ ID NO: 8 - protein, 736 aa, Artificial Sequence
  Synthetic Construct
MAADGYLPDWLEDNLSEGIREWWALKPGAPQPKANQQHQDNARGLVLPGYKYLGPGNGLDKGEPVNEADAAALEHDKAYDQQLKAGDNPYLKYNHADAEFQERLKEDTSFGGNLGRAVFQAKKRLLEPLGLVEEAAKTAPGKKRPVEQSPQEPDSSVGIGKSGAQPAKKRLNFGQTGDTESVPDPQPIGEPPAAPSGVGSLTMASGGGAPVADNNEGADGVGSSSGNWHCDSQWLGDRVITTSTRTWALPTYNNHLYKQISNSTSGGSSNDNAYFGYSTPWGYFDFNRFHCHFSPRDWQRLINNNWGFRPKRLNFKLFNIQVKEVTDNNGVKTIANNLTSTVQVFTDSDYQLPYVLGSAHEGCLPPFPADVFMIPQYGYLTLNDGSQAVGRSSFYCLEYFPSQMLRTGNNFQFSYEFENVPFHSSYAHSQSLDRLMNPLIDQYLYYLSKTINGSGQNQQTLKFSVAGPSNMAVQGRNYIPGPSYRQQRVSTTVTQNNNSEFAWPGASSWALNGRNSLMNPGPAMASHKEGEDRFFPLSGSLIFGKQGTGRDNVDADKVMITNEEEIKTTNPVATESYGQVATNHQSAQAQAQTGWVQNQGILPGMVWQDRDVYLQGPIWAKIPHTDGNFHPSPLMGGFGMKHPPPQILIKNTPVPADPPTAFNKDKLNSFITQYSTGQVSVEIEWELQKENSKRWNPEIQYTSNYYKSNNVEFAVNTEGVYSEPRPIGTRYLTRNL

SEQ ID NO: 9 - DNA, 1866 bp, Artificial Sequence
  AAVhu68 rep coding sequence
  CDS (1)..(1866)
atgccggggttttacgagattgtgattaaggtccccagcgaccttgacgagcatctgcccggcatttctgacagctttgtgaactgggtggccgagaaggaatgggagttgccgccagattctgacatggatctgaatctgattgagcaggcacccctgaccgtggccgagaagctgcagcgcgactttctgacggaatggcgccgtgtgagtaaggccccggaggctcttttctttgtgcaatttgagaagggagagagctacttccacatgcacgtgctcgtggaaaccaccggggtgaaatccatggttttgggacgtttcctgagtcagattcgcgaaaaactgattcagagaatttaccgcgggatcgagccgactttgccaaactggttcgcggtcacaaagaccagaaatggcgccggaggcgggaacaaggtggtggatgagtgctacatccccaattacttgctccccaaaacccagcctgagctccagtgggcgtggactaatatggaacagtatttaagcgcctgtttgaatctcacggagcgtaaacggttggtggcgcagcatctgacgcacgtgtcgcagacgcaggagcagaacaaagagaatcagaatcccaattctgatgcgccggtgatcagatcaaaaacttcagccaggtacatggagctggtcgggtggctcgtggacaaggggattacctcggagaagcagtggatccaggaggaccaggcctcatacatctccttcaatgcggcctccaactcgcggtcccaaatcaaggtcgccttggacaatgcgggaaagattatgagcctgactaaaaccgcccccgactacctggtgggccagcagcccgtggaggacatttccagcaatcggatttataaaattttggaactaaacgggtacgatccccaatatgcggcttccgtctttctgggatgggccacgaaaaagttcggcaagaggaacaccatctggctgtttgggcctgcaactaccgggaagaccaacatcgcggaggccatagcccacactgtgcccttctacgggtgcgtaaactggaccaatgagaactttcccttcaacgactgtgtcgacaagatggtgatctggtgggaggaggggaagatgaccgccaaggtcgtggagtcggccaaagccattctcggaggaagcaaggtgcgcgtggaccagaaatgcaagtcctcggcccagatagacccgactcccgtgatcgtcacctccaacaccaacatgtgcgccgtgattgacgggaactcaacgaccttcgaacaccagcagccgttgcaagaccggatgttcaaatttgaactcacccgccgtctggatcatgactttgggaaggtcaccaagcaggaagtcaaagactttttccggtgggcaaaggatcacgtggttgaggtggagcatgaattctacgtcaaaaagggtggagccaagaaaagacccgcccccagtgacgcagatataagtgagcccaaacgggtgcgcgagtcagttgcgcagccatcgacgtcagacgcggaagcttcgatcaactacgcggacaggtaccaaaacaaatgttctcgtcacgtgggcatgaatctgatgctgtttccctgcagacaatgcgagagactgaatcagaattcaaatatctgcttcactcacggtgtcaaagactgtttagagtgctttcccgtgtcagaatctcaacccgtttctgtcgtcaaaaaggcgtatcagaaactgtgctacattcatcacatcatgggaaaggtgccagacgcttgcactgcttgcgacctggtcaatgtggacttggatgactgtgtttctgaacaataa

SEQ ID NO: 10 - protein, 621 aa, Artificial Sequence
  Synthetic Construct
MPGFYEIVIKVPSDLDEHLPGISDSFVNWVAEKEWELPPDSDMDLNLIEQAPLTVAEKLQRDFLTEWRRVSKAPEALFFVQFEKGESYFHMHVLVETTGVKSMVLGRFLSQIREKLIQRIYRGIEPTLPNWFAVTKTRNGAGGGNKVVDECYIPNYLLPKTQPELQWAWTNMEQYLSACLNLTERKRLVAQHLTHVSQTQEQNKENQNPNSDAPVIRSKTSARYMELVGWLVDKGITSEKQWIQEDQASYISFNAASNSRSQIKVALDNAGKIMSLTKTAPDYLVGQQPVEDISSNRIYKILELNGYDPQYAASVFLGWATKKFGKRNTIWLFGPATTGKTNIAEAIAHTVPFYGCVNWTNENFPFNDCVDKMVIWWEEGKMTAKVVESAKAILGGSKVRVDQKCKSSAQIDPTPVIVTSNTNMCAVIDGNSTTFEHQQPLQDRMFKFELTRRLDHDFGKVTKQEVKDFFRWAKDHVVEVEHEFYVKKGGAKKRPAPSDADISEPKRVRESVAQPSTSDAEASINYADRYQNKCSRHVGMNLMLFPCRQCERLNQNSNICFTHGVKDCLECFPVSESQPVSVVKKAYQKLCYIHHIMGKVPDACTACDLVNVDLDDCVSEQ

SEQ ID NO: 11 - DNA, 1545 bp, Homo sapiens
ccacaaatgtgggagggcgataaccactcgtagaaagcgtgagaagttactacaagcggtcctcccggccaccgtactgttccgctcccagaagccccgggcggcggaagtcgtcactcttaagaagggacggggccccacgctgcgcacccgcgggtttgctatggcgatgagcagcggcggcagtggtggcggcgtcccggagcaggaggattccgtgctgttccggcgcggcacaggccagagcgatgattctgacatttgggatgatacagcactgataaaagcatatgataaagctgtggcttcatttaagcatgctctaaagaatggtgacatttgtgaaacttcgggtaaaccaaaaaccacacctaaaagaaaacctgctaagaagaataaaagccaaaagaagaatactgcagcttccttacaacagtggaaagttggggacaaatgttctgccatttggtcagaagacggttgcatttacccagctaccattgcttcaattgattttaagagagaaacctgtgttgtggtttacactggatatggaaatagagaggagcaaaatctgtccgatctactttccccaatctgtgaagtagctaataatatagaacaaaatgctcaagagaatgaaaatgaaagccaagtttcaacagatgaaagtgagaactccaggtctcctggaaataaatcagataacatcaagcccaaatctgctccatggaactcttttctccctccaccaccccccatgccagggccaagactgggaccaggaaagataattcccccaccacctcccatatgtccagattctcttgatgatgctgatgctttgggaagtatgttaatttcatggtacatgagtggctatcatactggctattatatgggtttcagacaaaatcaaaaagaaggaaggtgctcacattccttaaattaaggagaaatgctggcatagagcagcactaaatgacaccactaaagaaacgatcagacagatctggaatgtgaagcgttatagaagataactggcctcatttcttcaaaatatcaagtgttgggaaagaaaaaaggaagtggaatgggtaactcttcttgattaaaagttatgtaataaccaaatgcaatgtgaaatattttactggactctattttgaaaaaccatctgtaaaagactggggtgggggtgggaggccagcacggtggtgaggcagttgagaaaatttgaatgtggattagattttgaatgatattggataattattggtaattttatgagctgtgagaagggtgttgtagtttataaaagactgtcttaatttgcatacttaagcatttaggaatgaagtgttagagtgtcttaaaatgtttcaaatggtttaacaaaatgtatgtgaggcgtatgtggcaaaatgttacagaatctaactggtggacatggctgttcattgtactgtttttttctatcttctatatgtttaaaagtatataataaaaatatttaatttttttttaaaaaaaaaaaaaaaaaaa

SEQ ID NO: 12 - protein, 262 aa, Homo sapiens
MAMSSGGSGGGVPEQEDSVLFRRGTGQSDDSDIWDDTALIKAYDKAVASFKHALKNGDICETSGKPKTTPKRKPAKKNKSQKKNTAASLQQWKVGDKCSAIWSEDGCIYPATIASIDFKRETCVVVYTGYGNREEQNLSDLLSPICEVANNIEQNAQENENESQVSTDESENSRSPGNKSDNIKPKSAPWNSFLPPPPPMPGPRLGPGKIIPPPPPICPDSLDDADALGSMLISWYMSGYHTGYYMGFRQNQKEGRCSHSLN

SEQ ID NO: 13 - DNA, 1571 bp, Homo sapiens
ccacaaatgtgggagggcgataaccactcgtagaaagcgtgagaagttactacaagcggtcctcccggccaccgtactgttccgctcccagaagccccgggcggcggaagtcgtcactcttaagaagggacggggccccacgctgcgcacccgcgggtttgctatggcgatgagcagcggcggcagtggtggcggcgtcccggagcaggaggattccgtgctgttccggcgcggcacaggccagagcgatgattctgacatttgggatgatacagcactgataaaagcatatgataaagctgtggcttcatttaagcatgctctaaagaatggtgacatttgtgaaacttcgggtaaaccaaaaaccacacctaaaagaaaacctgctaagaagaataaaagccaaaagaagaatactgcagcttccttacaacagtggaaagttggggacaaatgttctgccatttggtcagaagacggttgcatttacccagctaccattgcttcaattgattttaagagagaaacctgtgttgtggtttacactggatatggaaatagagaggagcaaaatctgtccgatctactttccccaatctgtgaagtagctaataatatagaacaaaatgctcaagagaatgaaaatgaaagccaagtttcaacagatgaaagtgagaactccaggtctcctggaaataaatcagataacatcaagcccaaatctgctccatggaactcttttctccctccaccaccccccatgccagggccaagactgggaccaggaaagccaggtctaaaattcaatggcccaccaccgccaccgccaccaccaccaccccacttactatcatgctggctgcctccatttccttctggaccaccaataattcccccaccacctcccatatgtccagattctcttgatgatgctgatgctttgggaagtatgttaatttcatggtacatgagtggctatcatactggctattatatggaaatgctggcatagagcagcactaaatgacaccactaaagaaacgatcagacagatctggaatgtgaagcgttatagaagataactggcctcatttcttcaaaatatcaagtgttgggaaagaaaaaaggaagtggaatgggtaactcttcttgattaaaagttatgtaataaccaaatgcaatgtgaaatattttactggactctattttgaaaaaccatctgtaaaagactggggtgggggtgggaggccagcacggtggtgaggcagttgagaaaatttgaatgtggattagattttgaatgatattggataattattggtaattttatgagctgtgagaagggtgttgtagtttataaaagactgtcttaatttgcatacttaagcatttaggaatgaagtgttagagtgtcttaaaatgtttcaaatggtttaacaaaatgtatgtgaggcgtatgtggcaaaatgttacagaatctaactggtggacatggctgttcattgtactgtttttttctatcttctatatgtttaaaagtatataataaaaatatttaatttttttttaaa

SEQ ID NO: 14 - protein, 282 aa, Homo sapiens
MAMSSGGSGGGVPEQEDSVLFRRGTGQSDDSDIWDDTALIKAYDKAVASFKHALKNGDICETSGKPKTTPKRKPAKKNKSQKKNTAASLQQWKVGDKCSAIWSEDGCIYPATIASIDFKRETCVVVYTGYGNREEQNLSDLLSPICEVANNIEQNAQENENESQVSTDESENSRSPGNKSDNIKPKSAPWNSFLPPPPPMPGPRLGPGKPGLKFNGPPPPPPPPPPHLLSCWLPPFPSGPPIIPPPPPICPDSLDDADALGSMLISWYMSGYHTGYYMEMLA

SEQ ID NO: 15 - DNA, 3258 bp, Artificial Sequence
  AAV.CB7.CI.hSMN vector genome
  repeat_region (1)..(130): AAV2- 5'ITR
  promoter (197)..(579): CMV IE promoter
  promoter (582)..(863): CB promoter
  Intron (958)..(1930): CMV IE promoter
  misc_feature (1948)..(2829): hSMN coding sequence
  polyA_signal (2914)..(3040)
  repeat_region (3129)..(3258): AAV2- 3'ITR
ctgcgcgctcgctcgctcactgaggccgcccgggcaaagcccgggcgtcgggcgacctttggtcgcccggcctcagtgagcgagcgagcgcgcagagagggagtggccaactccatcactaggggttccttgtagttaatgattaacccgccatgctacttatctaccagggtaatggggatcctctagaactatagctagtcgacattgattattgactagttattaatagtaatcaattacggggtcattagttcatagcccatatatggagttccgcgttacataacttacggtaaatggcccgcctggctgaccgcccaacgacccccgcccattgacgtcaataatgacgtatgttcccatagtaacgccaatagggactttccattgacgtcaatgggtggactatttacggtaaactgcccacttggcagtacatcaagtgtatcatatgccaagtacgccccctattgacgtcaatgacggtaaatggcccgcctggcattatgcccagtacatgaccttatgggactttcctacttggcagtacatctacgtattagtcatcgctattaccatggtcgaggtgagccccacgttctgcttcactctccccatctcccccccctccccacccccaattttgtatttatttattttttaattattttgtgcagcgatgggggcggggggggggggggggcgcgcgccaggcggggcggggcggggcgaggggcggggcggggcgaggcggagaggtgcggcggcagccaatcagagcggcgcgctccgaaagtttccttttatggcgaggcggcggcggcggcggccctataaaaagcgaagcgcgcggcgggcggggagtcgctgcgacgctgccttcgccccgtgccccgctccgccgccgcctcgcgccgcccgccccggctctgactgaccgcgttactcccacaggtgagcgggcgggacggcccttctcctccgggctgtaattagcgcttggtttaatgacggcttgtttcttttctgtggctgcgtgaaagccttgaggggctccgggagggccctttgtgcggggggagcggctcggggggtgcgtgcgtgtgtgtgtgcgtggggagcgccgcgtgcggctccgcgctgcccggcggctgtgagcgctgcgggcgcggcgcggggctttgtgcgctccgcagtgtgcgcgaggggagcgcggccgggggcggtgccccgcggtgcggggggggctgcgaggggaacaaaggctgcgtgcggggtgtgtgcgtgggggggtgagcagggggtgtgggcgcgtcggtcgggctgcaaccccccctgcacccccctccccgagttgctgagcacggcccggcttcgggtgcggggctccgtacggggcgtggcgcggggctcgccgtgccgggcggggggtggcggcaggtgggggtgccgggcggggcggggccgcctcgggccggggagggctcgggggaggggcgcggcggcccccggagcgccggcggctgtcgaggcgcggcgagccgcagccattgccttttatggtaatcgtgcgagagggcgcagggacttcctttgtcccaaatctgtgcggagccgaaatctgggaggcgccgccgcaccccctctagcgggcgcggggcgaagcggtgcggcgccggcaggaaggaaatgggcggggagggccttcgtgcgtcgccgcgccgccgtccccttctccctctccagcctcggggctgtccgcggggggacggctgccttcgggggggacggggcagggcggggttcggcttctggcgtgtgaccggcggctctagagcctctgctaaccatgttcatgccttcttctttttcctacagctcctgggcaacgtgctggttattgtgctgtctcatcattttggcaaagaattctagcttgccaccatggccatgtcgagtgggggcagtggagggggagtgccagaacaggaagattccgtgctgttcaggcgaggaaccgggcagagtgacgacagtgacatttgggacgacacggccctgatcaaggcctatgacaaagccgtggcctccttcaagcacgcgctgaagaacggcgacatttgcgaaaccagcggcaagcctaagaccacccctaaacggaagcccgccaagaaaaataagtcccagaaaaagaacacagccgcaagtcttcagcaatggaaggtgggggataagtgctccgcgatatggagtgaagacgggtgcatctatcctgccaccatcgccagcatagacttcaagcgcgaaacctgcgtggtggtgtacactggatacgggaaccgggaggagcagaacctgagcgacctgttgagccctatttgtgaggtggccaacaacatcgagcagaatgcgcaagaaaatgaaaacgagagtcaggtgtccaccgatgagagtgaaaacagtaggagccccggcaacaaatccgacaatatcaagcccaaaagcgcaccctggaatagcttccttccacccccccccccaatgcccggacctcgactgggccccggaaagcctggcctgaagttcaacggcccccctcctcctcctccccctcctcccccccacctgctgagctgctggttgccccctttcccttcgggaccccctatcatacctccccccccccctatttgccctgactccctggacgacgcggacgcgctgggcagtatgctcatctcgtggtacatgtcaggataccacaccgggtactacatgggcttcagacaaaatcagaaggaaggacgatgtagtcactccctgaattaatgatagctagaattcacgcgtggtacctctagagtcgacccgggcggcctcgaggacggggtgaactacgcctgaggatccgatctttttccctctgccaaaaattatggggacatcatgaagccccttgagcatctgacttctggctaataaaggaaatttattttcattgcaatagtgtgttggaattttttgtgtctctcactcggaagcaattcgttgatctgaatttcgaccacccataatacccattaccctggtagataagtagcatggcgggttaatcattaactacaaggaacccctagtgatggagttggccactccctctctgcgcgctcgctcgctcactgaggccgggcgaccaaaggtcgcccgacgcccgggctttgcccgggcggcctcagtgagcgagcgagcgcgcag

SEQ ID NO: 16 - protein, 736 aa, Artificial Sequence
  Encoded AAV9 vp1 amino acid sequence
  MISC_FEATURE (1)..(137): encoded vp1-unique region
  MISC_FEATURE (1)..(736): encoded vp1 amino acid sequence
  MISC_FEATURE (1)..(736): encoded vp1 amino acid sequence
  MISC_FEATURE (138)..(736): encoded amino acid sequence of alternative splice variant vp2 protein
  MISC_FEATURE (203)..(736): encoded amino acid sequence of alternative splice variant vp3 protein
MAADGYLPDWLEDNLSEGIREWWALKPGAPQPKANQQHQDNARGLVLPGYKYLGPGNGLDKGEPVNAADAAALEHDKAYDQQLKAGDNPYLKYNHADAEFQERLKEDTSFGGNLGRAVFQAKKRLLEPLGLVEEAAKTAPGKKRPVEQSPQEPDSSAGIGKSGAQPAKKRLNFGQTGDTESVPDPQPIGEPPAAPSGVGSLTMASGGGAPVADNNEGADGVGSSSGNWHCDSQWLGDRVITTSTRTWALPTYNNHLYKQISNSTSGGSSNDNAYFGYSTPWGYFDFNRFHCHFSPRDWQRLINNNWGFRPKRLNFKLFNIQVKEVTDNNGVKTIANNLTSTVQVFTDSDYQLPYVLGSAHEGCLPPFPADVFMIPQYGYLTLNDGSQAVGRSSFYCLEYFPSQMLRTGNNFQFSYEFENVPFHSSYAHSQSLDRLMNPLIDQYLYYLSKTINGSGQNQQTLKFSVAGPSNMAVQGRNYIPGPSYRQQRVSTTVTQNNNSEFAWPGASSWALNGRNSLMNPGPAMASHKEGEDRFFPLSGSLIFGKQGTGRDNVDADKVMITNEEEIKTTNPVATESYGQVATNHQSAQAQAQTGWVQNQGILPGMVWQDRDVYLQGPIWAKIPHTDGNFHPSPLMGGFGMKHPPPQILIKNTPVPADPPTAFNKDKLNSFITQYSTGQVSVEIEWELQKENSKRWNPEIQYTSNYYKSNNVEFAVNTEGVYSEPRPIGTRYLTRNL

SEQ ID NO: 17 - protein, 738 aa, Artificial Sequence
  Encoded AAVrh10 vp1 amino acid sequence
MAADGYLPDWLEDNLSEGIREWWDLKPGAPKPKANQQKQDDGRGLVLPGYKYLGPFNGLDKGEPVNAADAAALEHDKAYDQQLKAGDNPYLRYNHADAEFQERLQEDTSFGGNLGRAVFQAKKRVLEPLGLVEEGAKTAPGKKRPVEPSPQRSPDSSTGIGKKGQQPAKKRLNFGQTGDSESVPDPQPIGEPPAGPSGLGSGTMAAGGGAPMADNNEGADGVGSSSGNWHCDSTWLGDRVITTSTRTWALPTYNNHLYKQISNGTSGGSTNDNTYFGYSTPWGYFDFNRFHCHFSPRDWQRLINNNWGFRPKRLNFKLFNIQVKEVTQNEGTKTIANNLTSTIQVFTDSEYQLPYVLGSAHQGCLPPFPADVFMIPQYGYLTLNNGSQAVGRSSFYCLEYFPSQMLRTGNNFEFSYQFEDVPFHSSYAHSQSLDRLMNPLIDQYLYYLSRTQSTGGTAGTQQLLFSQAGPNNMSAQAKNWLPGPCYRQQRVSTTLSQNNNSNFAWTGATKYHLNGRDSLVNPGVAMATHKDDEERFFPSSGVLMFGKQGAGKDNVDYSSVMLTSEEEIKTTNPVATEQYGVVADNLQQQNAAPIVGAVNSQGALPGMVWQNRDVYLQGPIWAKIPHTDGNFHPSPLMGGFGLKHPPPQILIKNTPVPADPPTTFSQAKLASFITQYSTGQVSVEIEWELQKENSKRWNPEIQYTSNYYKSTNVDFAVNTDGTYSEPRPIGTRYLTRNL

SEQ ID NO: 18 - protein, 736 aa, Artificial Sequence
  Encoded AAVhu31 vp1 amino acid sequence
MAADGYLPDWLEDTLSEGIRQWWKLKPGPPPPKPAERHKDDSRGLVLPGYKYLGPGNGLDKGEPVNAADAAALEHDKAYDQQLKAGDNPYLKYNHADAEFQERLKEDTSFGGNLGRAVFQAKKRLLEPLGLVEEAAKTAPGKKRPVEQSPQEPDSSAGIGKSGSQPAKKKLNFGQTGDTESVPDPQPIGEPPAAPSGVGSLTMASGGGAPVADNNEGADGVGSSSGNWHCDSQWLGDRVITTSTRTWALPTYNNHLYKQISNSTSGGSSNDNAYFGYSTPWGYFDFNRFHCHFSPRDWQRLINNNWGFRPKRLNFKLFNIQVKEVTDNNGVKTIANNLTSTVQVFTDSDYQLPYVLGSAHEGCLPPFPADVFMIPQYGYLTLNDGGQAVGRSSFYCLEYFPSQMLRTGNNFQFSYEFENVPFHSSYAHSQSLDRLMNPLIDQYLYYLSKTINGSGQNQQTLKFSVAGPSNMAVQGRNYIPGPSYRQQRVSTTVTQNNNSEFAWPGASSWALNGRNSLMNPGPAMASHKEGEDRFFPLSGSLIFGKQGTGRDNVDADKVMITNEEEIKTTNPVATESYGQVATNHQSAQAQAQTGWVQNQGILPGMVWQDRDVYLQGPIWAKIPHTDGNFHPSPLMGGFGMKHPPPQILIKNTPVPADPPTAFNKDKLNSFITQYSTGQVSVEIEWELQKENSKRWNPEIQYTSNYYKSNNVEFAVSTEGVYSEPRPIGTRYLTRNL

SEQ ID NO: 19 - protein, 736 aa, Artificial Sequence
  Encoded AAVhu32 vp1 amino acid sequence
MAADGYLPDWLEDTLSEGIRQWWKLKPGPPPPKPAERHKDDSRGLVLPGYKYLGPGNGLDKGEPVNAADAAALEHDKAYDQQLKAGDNPYLKYNHADAEFQERLKEDTSFGGNLGRAVFQAKKRLLEPLGLVEEAAKTAPGKKRPVEQSPQEPDSSAGIGKSGSQPAKKKLNFGQTGDTESVPDPQPIGEPPAAPSGVGSLTMASGGGAPVADNNEGADGVGSSSGNWHCDSQWLGDRVITTSTRTWALPTYNNHLYKQISNSTSGGSSNDNAYFGYSTPWGYFDFNRFHCHFSPRDWQRLINNNWGFRPKRLNFKLFNIQVKEVTDNNGVKTIANNLTSTVQVFTDSDYQLPYVLGSAHEGCLPPFPADVFMIPQYGYLTLNDGSQAVGRSSFYCLEYFPSQMLRTGNNFQFSYEFENVPFHSSYAHSQSLDRLMNPLIDQYLYYLSKTINGSGQNQQTLKFSVAGPSNMAVQGRNYIPGPSYRQQRVSTTVTQNNNSEFAWPGASSWALNGRNSLMNPGPAMASHKEGEDRFFPLSGSLIFGKQGTGRDNVDADKVMITNEEEIKTTNPVATESYGQVATNHQSAQAQAQTGWVQNQGILPGMVWQDRDVYLQGPIWAKIPHTDGNFHPSPLMGGFGMKHPPPQILIKNTPVPADPPTAFNKDKLNSFITQYSTGQVSVEIEWELQKENSKRWNPEIQYTSNYYKSNNVEFAVNTEGVYSEPRPIGTRYLTRNL

SEQ ID NO: 20 - DNA, 2211 bp, Artificial Sequence
  AAVhu31 vp1 coding sequence
atggctgccgatggttatcttccagattggctcgaggacaaccttagtgaaggaattcgcgagtggtgggctttgaaacctggagcccctcaacccaaggcaaatcaacaacatcaagacaacgctcgaggtcttgtgcttccgggttacaaataccttggacccggcaacggactcgacaagggggagccggtcaacgcagcagacgcggcggccctcgagcacgacaaggcctacgaccagcagctcaaggccggagacaacccgtacctcaagtacaaccacgccgacgccgagttccaggagcggctcaaagaagatacgtcttttgggggcaacctcgggcgagcagtcttccaggccaaaaagaggcttcttgaacctcttggtctggttgaggaagcggctaagacggctcctggaaagaagaggcctgtagagcagtctcctcaggaaccggactcctccgcgggtattggcaaatcgggtgcacagcccgctaaaaagagactcaatttcggtcagactggcgacacagagtcagtcccagaccctcaaccaatcggagaacctcccgcagccccctcaggtgtgggatctcttacaatggcttcaggtggtggcgcaccagtggcagacaataacgaaggtgccgatggagtgggtagttcctcgggaaattggcattgcgattcccaatggctgggggacagagtcatcaccaccagcacccgaacctgggccctgcccacctacaacaatcacctctacaagcaaatctccaacagcacatctggaggatcttcaaatgacaacgcctacttcggctacagcaccccctgggggtattttgacttcaacagattccactgccacttctcaccacgtgactggcagcgactcatcaacaacaactggggattccggcctaagcgactcaacttcaagctcttcaacattcaggtcaaagaggttacggacaacaatggagtcaagaccatcgccaataaccttaccagcacggtccaggtcttcacggactcagactatcagctcccgtacgtgctcgggtcggctcacgagggctgcctcccgccgttcccagcggacgttttcatgattcctcagtacgggtatctgacgcttaatgatggaagccaggccgtgggtcgttcgtccttttactgcctggaatatttcccgtcgcaaatgctaagaacgggtaacaacttccagttcagctacgagtttgagaacgtacctttccatagcagctacgctcacagccaaagcctggaccgactaatgaatccactcatcgaccaatacttgtactatctctcaaagactattaacggttctggacagaatcaacaaacgctaaaattcagtgtggccggacccagcaacatggctgtccagggaagaaactacatacctggacccagctaccgacaacaacgtgtctcaaccactgtgactcaaaacaacaacagcgaatttgcttggcctggagcttcttcttgggctctcaatggacgtaatagcttgatgaatcctggacctgctatggccagccacaaagaaggagaggaccgtttctttcctttgtctggatctttaatttttggcaaacaaggaactggaagagacaacgtggatgcggacaaagtcatgataaccaacgaagaagaaattaaaactactaacccggtagcaacggagtcctatggacaagtggccacaaaccaccagagtgcccaagcacaggcgcagaccggctgggttcaaaaccaaggaatacttccgggtatggtttggcaggacagagatgtgtacctgcaaggacccatttgggccaaaattcctcacacggacggcaactttcacccttctccgctgatgggagggtttggaatgaagcacccgcctcctcagatcctcatcaaaaacacacctgtacctgcggatcctccaacggccttcaacaaggacaagctgaactctttcatcacccagtattctactggccaagtcagcgtggagatcgagtgggagctgcagaaggaaaacagcaagcgctggaacccggagatccagtacacttccaactattacaagtctaataatgttgaatttgctgttaatactgaaggtgtatatagtgaaccccgccccattggcaccagatacctgactcgtaatctgtaa

SEQ ID NO: 21 - DNA, 2211 bp, Artificial Sequence
  AAVhu32 vp1 coding sequence
atggctgccgatggttatcttccagattggctcgaggacactctctctgaaggaataagacagtggtggaagctcaaacctggcccaccaccaccaaagcccgcagagcggcataaggacgacagcaggggtcttgtgcttcctgggtacaagtacctcggacccggcaacggactcgacaagggggagccggtcaacgcagcagacgcggcggccctcgagcacgacaaggcctacgaccagcagctcaaggccggagacaacccgtacctcaagtacaaccacgccgacgccgagttccaggagcggctcaaagaagatacgtcttttgggggcaacctcgggcgagcagtcttccaggccaaaaagaggcttcttgaacctcttggtctggttgaggaagcggctaagacggctcctggaaagaagaggcctgtagagcagtctcctcaggaaccggactcctccgcgggtattggcaaatcgggttcacagcccgctaaaaagaaactcaatttcggtcagactggcgacacagagtcagtccccgaccctcaaccaatcggagaacctcccgcagccccctcaggtgtgggatctcttacaatggcttcaggtggtggcgcaccagtggcagacaataacgaaggtgccgatggagtgggtagttcctcgggaaattggcattgcgattcccaatggctgggggacagagtcatcaccaccagcacccgaacctgggccctgcccacctacaacaatcacctctacaagcaaatctccaacagcacatctggaggatcttcaaatgacaacgcctacttcggctacagcaccccctgggggtattttgacttcaacagattccactgccacttctcaccacgtgactggcagcgactcatcaacaacaactggggattccggcctaagcgactcaacttcaagctcttcaacattcaggtcaaagaggttacggacaacaatggagtcaagaccatcgccaataaccttaccagcacggtccaggtcttcacggactcagactatcagctcccgtacgtgctcgggtcggctcacgagggctgcctcccgccgttcccagcggacgttttcatgattcctcagtacgggtatctgacgcttaatgatgggagccaggccgtgggtcgttcgtccttttactgcctggaatatttcccgtcgcaaatgctaagaacgggtaacaacttccagttcagctacgagtttgagaacgtacctttccatagcagctacgctcacagccaaagcctggaccgactaatgaatccactcatcgaccaatacttgtactatctctcaaagactattaacggttctggacagaatcaacaaacgctaaaattcagcgtggccggacccagcaacatggctgtccagggaagaaactacatacctggacccagctaccgacaacaacgtgtctcaaccactgtgactcaaaacaacaacagcgaatttgcttggcctggagcttcttcttgggctctcaatggacgtaatagcttgatgaatcctggacctgctatggccagccacaaagaaggagaggaccgtttctttcctttgtctggatctttaatttttggcaaacaaggaactggaagagacaacgtggatgcggacaaagtcatgataaccaacgaagaagaaattaaaactactaacccggtagcaacggagtcctatggacaagtggccacaaaccaccagagtgcccaagcacaggcgcagaccggctgggttcaaaaccaaggaatacttccgggtatggtttggcaggacagagatgtgtacctgcaaggacccatttgggccaaaattcctcacacggacggcaactttcacccttctccgctaatgggagggtttggaatgaagcacccgcctcctcagatcctcatcaaaaacacacctgtacctgcggatcctccaacggctttcaataaggacaagctgaactctttcatcacccagtattctactggccaagtcagcgtggagattgagtgggagctgcagaaggaaaacagcaagcgctggaacccggagatccagtacacttccaactattacaagtctaataatgttgaatttgctgttaatactgaaggtgtatatagtgaaccccgccccattggcaccagatacctgactcgtaatctgtaa

SEQ ID NO: 22 - DNA, 2211 bp, Artificial Sequence; identical to SEQ ID NO: 20
  AAV9 vp1 coding sequence

SEQ ID NO: 23 - DNA, 26 bp, Artificial Sequence
  Primer prm504
gctgcgtcaactggaccaatgagaac

SEQ ID NO: 24 - DNA, 28 bp, Artificial Sequence
  Primer prm505
cgcagagaccaaagttcaactgaaacga

SEQ ID NO: 25 - DNA, 3256 bp, Artificial Sequence
  AAV.CB7.CI.hSMN vector genome
  repeat_region (1)..(130): 5'ITR
  promoter (198)..(579): CMV IE promoter
  promoter (582)..(862): CB promoter
  TATA_signal (836)..(839)
  Intron (956)..(1928): Chicken beta-actin intron
  misc_feature (1946)..(2827): hSMN coding sequence
  polyA_signal (2912)..(3038): Rabbit globin polyA
  repeat_region (3127)..(3256): 3'ITR
ctgcgcgctcgctcgctcactgaggccgcccgggcaaagcccgggcgtcgggcgacctttggtcgcccggcctcagtgagcgagcgagcgcgcagagagggagtggccaactccatcactaggggttccttgtagttaatgattaacccgccatgctacttatctaccagggtaatggggatcctctagaactatagctagtcgacattgattattgactagttattaatagtaatcaattacggggtcattagttcatagcccatatatggagttccgcgttacataacttacggtaaatggcccgcctggctgaccgcccaacgacccccgcccattgacgtcaataatgacgtatgttcccatagtaacgccaatagggactttccattgacgtcaatgggtggagtatttacggtaaactgcccacttggcagtacatcaagtgtatcatatgccaagtacgccccctattgacgtcaatgacggtaaatggcccgcctggcattatgcccagtacatgaccttatgggactttcctacttggcagtacatctacgtattagtcatcgctattaccatggtcgaggtgagccccacgttctgcttcactctccccatctcccccccctccccacccccaattttgtatttatttattttttaattattttgtgcagcgatgggggcggggggggggggggggcgcgcgccaggcggggcggggcggggcgaggggcggggcggggcgaggcggagaggtgcggcggcagccaatcagagcggcgcgctccgaaagtttccttttatggcgaggcggcggcggcggcggccctataaaaagcgaagcgcgcggcgggcgggagtcgctgcgcgctgccttcgccccgtgccccgctccgccgccgcctcgcgccgcccgccccggctctgactgaccgcgttactcccacaggtgagcgggcgggacggcccttctcctccgggctgtaattagcgcttggtttaatgacggcttgtttcttttctgtggctgcgtgaaagccttgaggggctccgggagggccctttgtgcggggggagcggctcggggggtgcgtgcgtgtgtgtgtgcgtggggagcgccgcgtgcggctccgcgctgcccggcggctgtgagcgctgcgggcgcggcgcggggctttgtgcgctccgcagtgtgcgcgaggggagcgcggccgggggcggtgccccgcggtgcggggggggctgcgaggggaacaaaggctgcgtgcggggtgtgtgcgtgggggggtgagcagggggtgtgggcgcgtcggtcgggctgcaaccccccctgcacccccctccccgagttgctgagcacggcccggcttcgggtgcggggctccgtacggggcgtggcgcggggctcgccgtgccgggcggggggtggcggcaggtgggggtgccgggcggggcggggccgcctcgggccggggagggctcgggggaggggcgcggcggcccccggagcgccggcggctgtcgaggcgcggcgagccgcagccattgccttttatggtaatcgtgcgagagggcgcagggacttcctttgtcccaaatctgtgcggagccgaaatctgggaggcgccgccgcaccccctctagcgggcgcggggcgaagcggtgcggcgccggcaggaaggaaatgggcggggagggccttcgtgcgtcgccgcgccgccgtccccttctccctctccagcctcggggctgtccgcggggggacggctgccttcgggggggacggggcagggcggggttcggcttctggcgtgtgaccggcggctctagagcctctgctaaccatgttcatgccttcttctttttcctacagctcctgggcaacgtgctggttattgtgctgtctcatcattttggcaaagaattctagcttgccaccatggccatgtcgagtgggggcagtggagggggagtgccagaacaggaagattccgtgctgttcaggcgaggaaccgggcagagtgacgacagtgacatttgggacgacacggccctgatcaaggcctatgacaaagccgtggcctccttcaagcacgcgctgaagaacggcgacatttgcgaaaccagcggcaagcctaagaccacccctaaacggaagcccgccaagaaaaataagtcccagaaaaagaacacagccgcaagtcttcagcaatggaaggtgggggataagtgctccgcgatatggagtgaagacgggtgcatctatcctgccaccatcgccagcatagacttcaagcgcgaaacctgcgtggtggtgtacactggatacgggaaccgggaggagcagaacctgagcgacctgttgagccctatttgtgaggtggccaacaacatcgagcagaatgcgcaagaaaatgaaaacgagagtcaggtgtccaccgatgagagtgaaaacagtaggagccccggcaacaaatccgacaatatcaagcccaaaagcgcaccctggaatagcttccttccacccccccccccaatgcccggacctcgactgggccccggaaagcctggcctgaagttcaacggcccccctcctcctcctccccctcctcccccccacctgctgagctgctggttgccccctttcccttcgggaccccctatcatacctccccccccccctatttgccctgactccctggacgacgcggacgcgctgggcagtatgctcatctcgtggtacatgtcaggataccacaccgggtactacatgggcttcagacaaaatcagaaggaaggacgatgtagtcactccctgaattaatgatagctagaattcacgcgtggtacctctagagtcgacccgggcggcctcgaggacggggtgaactacgcctgaggatccgatctttttccctctgccaaaaattatggggacatcatgaagccccttgagcatctgacttctggctaataaaggaaatttattttcattgcaatagtgtgttggaattttttgtgtctctcactcggaagcaattcgttgatctgaatttcgaccacccataatacccattaccctggtagataagtagcatggcgggttaatcattaactacaaggaacccctagtgatggagttggccactccctctctgcgcgctcgctcgctcactgaggccgggcgaccaaaggtcgcccgacgcccgggctttgcccgggcggcctcagtgagcgagcgagcgcgcag

SEQ ID NO: 26 - protein, 736 aa, Artificial Sequence
  modified hu68vp1
  MISC_FEATURE (23)..(23): Xaa may be W (Trp, tryptophan), or oxidated W.
  MISC_FEATURE (35)..(35): Xaa may be Asn, or deamidated to Asp, isoAsp, or Asp/isoAsp
  MISC_FEATURE (57)..(57): Xaa may be Asn, or deamidated to Asp, isoAsp, or Asp/isoAsp
  MISC_FEATURE (66)..(66): Xaa may be Asn, or deamidated to Asp, isoAsp, or Asp/isoAsp
  MISC_FEATURE (94)..(94): Xaa may be Asn, or deamidated to Asp, isoAsp, or Asp/isoAsp
  MISC_FEATURE (97)..(97): Xaa may be D (asp, aspartic acid), or isomerized D.
  MISC_FEATURE (107)..(107): Xaa may be D (asp, aspartic acid), or isomerized D.
  misc_feature (113)..(113): Xaa can be any naturally occurring amino acid
  MISC_FEATURE (149)..(149): Xaa may be S (Ser, serine), or Phosphorilated S
  MISC_FEATURE (149)..(149): Xaa may be S (Ser, serine), or Phosphorylated S
  MISC_FEATURE (247)..(247): Xaa may be W (Trp, tryptophan), or oxidated W (e.g., kynurenine).
  MISC_FEATURE (253)..(253): Xaa may be Asn, or deamidated to Asp, isoAsp, or Asp/isoAsp
  MISC_FEATURE (259)..(259): Xaa represents Q, or Q deamidated to glutamic acid (alpha-glutamic acid), gamma-glutamic acid (Glu), or a blend of alpha- and gamma-glutamic acid
  MISC_FEATURE (270)..(270): Xaa may be Asn, or deamidated to Asp, isoAsp, or Asp/isoAsp
  MISC_FEATURE (297)..(297): Xaa represents D (Asp, aspartic acid) or amindated D to N (Asn, asparagine)
  MISC_FEATURE (304)..(304): Xaa may be Asn, or deamidated to Asp, isoAsp, or Asp/isoAsp
  MISC_FEATURE (306)..(306): Xaa may be W (Trp, tryptophan), or oxidated W (e.g., kynurenine).
  MISC_FEATURE (314)..(314): Xaa may be Asn, or deamidated to Asp, isoAsp, or Asp/isoAsp
  MISC_FEATURE (319)..(319): Xaa may be Asn, or deamidated to Asp, isoAsp, or Asp/isoAsp
  MISC_FEATURE (329)..(329): Xaa may be Asn, or deamidated to Asp, isoAsp, or Asp/isoAsp
  MISC_FEATURE (332)..(332): Xaa may be K (lys, lysine), or acetylated K
  MISC_FEATURE (336)..(336): Xaa may be Asn, or deamidated to Asp, isoAsp, or Asp/isoAsp
  MISC_FEATURE (384)..(384): Xaa may be D (asp, aspartic acid), or isomerized D.
  MISC_FEATURE (404)..(404): Xaa may be M (Met, Methionine), or oxidated M.
  MISC_FEATURE (409)..(409): Xaa may be Asn, or deamidated to Asp, isoAsp, or Asp/isoAsp
  MISC_FEATURE (436)..(436): Xaa may be M (Met, Methionine), or oxidated M.
  MISC_FEATURE (452)..(452): Xaa may be Asn, or deamidated to Asp, isoAsp, or Asp/isoAsp
  MISC_FEATURE (477)..(477): Xaa may be Asn, or deamidated to Asp, isoAsp, or Asp/isoAsp
  MISC_FEATURE (499)..(499): Xaa may be S (Ser, serine), or Phosphorylated S
  MISC_FEATURE (512)..(512): Xaa may be Asn, or deamidated to Asp, isoAsp, or Asp/isoAsp
  MISC_FEATURE (515)..(515): Xaa may be Asn, or deamidated to Asp, isoAsp, or Asp/isoAsp
  MISC_FEATURE (518)..(518): Xaa may be M (Met, Methionine), or oxidated M.
  MISC_FEATURE (524)..(524): Xaa may be M (Met, Methionine), or oxidated M.
  MISC_FEATURE (559)..(559): Xaa may be M (Met, Methionine), or oxidated M.
  MISC_FEATURE (569)..(569): Xaa may be T (Thr, threonine), or Phosphorylated T
  MISC_FEATURE (586)..(586): Xaa may be S (Ser, serine), or Phosphorylated S
  MISC_FEATURE (599)..(599): Xaa represents Q, or Q deamidated to glutamic acid (alpha-glutamic acid), gamma-glutamic acid (Glu), or a blend of alpha- and gamma-glutamic acid
  MISC_FEATURE (605)..(605): Xaa may be M (Met, Methionine), or oxidated M.
  MISC_FEATURE (619)..(619): Xaa may be W (Trp, tryptophan), or oxidated W (e.g., kynurenine).
  MISC_FEATURE (628)..(628): Xaa may be Asn, or deamidated to Asp, isoAsp, or Asp/isoAsp
  MISC_FEATURE (640)..(640): Xaa may be M (Met, Methionine), or oxidated M.
  MISC_FEATURE (651)..(651): Xaa may be Asn, or deamidated to Asp, isoAsp, or Asp/isoAsp
  MISC_FEATURE (663)..(663): Xaa may be Asn, or deamidated to Asp, isoAsp, or Asp/isoAsp
  MISC_FEATURE (666)..(666): Xaa may be K (lys, lysine), or acetylated K
  MISC_FEATURE (689)..(689): Xaa may be K (lys, lysine), or acetylated K
  MISC_FEATURE (693)..(693): Xaa may be K (lys, lysine), or acetylated K
  MISC_FEATURE (695)..(695): Xaa may be W (Trp, tryptophan), or oxidated W.
  MISC_FEATURE (709)..(709): Xaa may be Asn, or deamidated to Asp, isoAsp, or Asp/isoAsp
  MISC_FEATURE (735)..(735): Xaa may be Asn, or deamidated to Asp, isoAsp, or Asp/isoAsp
MAADGYLPDWLEDNLSEGIREWXALKPGAPQPKAXQQHQDNARGLVLPGYKYLGPGXGLDKGEPVXEADAAALEHDKAYDQQLKAGDNPYLKYXHAXAEFQERLKEXTSFGGXLGRAVFQAKKRLLEPLGLVEEAAKTAPGKKRPVEQXPQEPDSSVGIGKSGAQPAKKRLNFGQTGDTESVPDPQPIGEPPAAPSGVGSLTMASGGGAPVADNNEGADGVGSSSGNWHCDSQWLGDRVITTSTRTXALPTYXNHLYKXISNSTSGGSSXDNAYFGYSTPWGYFDFNRFHCHFSPRXWQRLINXNXGFRPKRLXFKLFXIQVKEVTDNXGVXTIAXNLTSTVQVFTDSDYQLPYVLGSAHEGCLPPFPADVFMIPQYGYLTLNXGSQAVGRSSFYCLEYFPSQXLRTGXNFQFSYEFENVPFHSSYAHSQSLDRLXNPLIDQYLYYLSKTIXGSGQNQQTLKFSVAGPSNMAVQGRXYIPGPSYRQQRVSTTVTQNNNXEFAWPGASSWALXGRXSLXNPGPAXASHKEGEDRFFPLSGSLIFGKQGTGRDNVDADKVXITNEEEIKTXNPVATESYGQVATNHQXAQAQAQTGWVQNQGILPGXVWQDRDVYLQGPIXAKIPHTDGXFHPSPLMGGFGXKHPPPQILIKXTPVPADPPTAFXKDXLNSFITQYSTGQVSVEIEWELQXENSXRXNPEIQYTSNYYKSXNVEFAVNTEGVYSEPRPIGTRYLTRXL